European Patent Specification EP 3 864 656 B1, published August 20, 2025. Title: METHODS AND SYSTEMS FOR EVALUATING MICROSATELLITE INSTABILITY STATUS. Applicant: LIFE TECHNOLOGIES CORPORATION EL-DIFRAWY, Sameh. The sequence listing filed with the application follows.

SEQUENCE LISTING (2 sequences)

SEQ ID NO: 1 - DNA, 19 bp, Artificial Sequence
  Synthetic
acgtcaaaaaaaaaaggtc

SEQ ID NO: 2 - DNA, 15 bp, Artificial Sequence
  Synthetic
acgtcaaaaaaggtc